European Patent Specification EP 3 713 586 B1, published January 4, 2023. Title: VIBRIO SP. ORGANISMS WITH MODIFIED LIPOPOLYSACCHARIDE. Applicant: SYNTHETIC GENOMICS, INC. WEINSTOCK, Matthew T GIBSON , Daniel G. STRIMLING, Daniel. The sequence listing filed with the application follows.

SEQUENCE LISTING (4 sequences)

SEQ ID NO: 1 - DNA, 975 bp, Vibrio natriegens
  misc_feature: lpxL
atgggcacatctggcgattctttcatgaacaaacaaaaagagcctgttttcgaggctcggttcctaatgcctcggtactggggaactctactcatcatcggggtgatgtatttacttagccttctacctttcaaatttcaattattcctgggacgcagtattggccgtttggccatgcgattaatgaaaaagcgtcaggtcaccattcgtcgcaatttagagctctgcttcccgaagatggacgagagcaaacgagaagcgatactgaaagctaacatcgataattctggcattgcactgtttgagacagcgatggcttggttctggccggatcgcagggttaataaacacgtaacgataaaagggatggaacacctagaagcgttagaaaaagacggcaaaggggtgttgatgcttgccgttcattccatgaacttagagctgggtgcacgtgcatttggcattcaaaaatctggaatgggtgtttatcgaccgaataacaatccttgttttgactattttcagtacaagggtcgttcgcgttccaatcgtactttgatcgatcgtaaaaatgttagaggaatgctggacgctttgaattccggcaatcgcgtttggtatgcgcctgaccatgattatggaaccagaagatcgacctttgcgcctttgtttgctgtcaaaaacgcctgtaccacaacaggcaccagtttacttgttgatgcaacagattgtgcgattgtgccgtttaccatggtaagaggggatgatggccattacacattaacgatcagggagccagttgacggatttcctaaaggtgataccagaaacgcggcgatttttatcaataaaattgttgaagagtcgattatggctagccctagtcaatacatgtggttgcaccgccgatttaaaaccagaccgcaaggtgaagattgtttgtacaatcctcagttaatccctgcgatgagttag

SEQ ID NO: 2 - DNA, 981 bp, Vibrio natriegens
  misc_feature: lpxM
atgatcaataaacgtgatgatttcgatcccaaagcctataaccctgagtttgaccgctcatttctcaagcctaaatattggggaacctggctcgctgtttttagctcaatttttatcgcattgctgcccctcgcttttcaccagtggctggcaaaagtgctggcatcacgtttagttaaatctaaagcaaactcagtcaacaacgtaaagaccaacttagccttgtgtttcccacagttaagtgaacaagagcgtgaccaactggtttacaaaacgctttatactgccggcgtatttactcttagatttggcttggtctctttgcgttcacccgaatggctgcaatcaaagtgtgactttgtaaactccgaacagttgctcgacctaactgagcaaaatcaaaaagtgattttattagtgccgcactcttggtcgattgatatacctgcggtactacttgcctcacaaggcttacctgtttctgcgatggcgaaaagacagaaaaacccagtaacagactggctaatgcatcgccaacgcgtgcaatatggtggccgtgtgtacgaacgctctggagggattaaacccttcatcaaatcgattaaagacggttacttgggctactatctaccagaccaggatcatggtgctgaactcagtgaatttgtggactttttcgcgacgacgaaggcaaccctgccaggtctgacaaaactggcgaaactgtcaaagtccaaagtaatcccgacttttgcctcactggatccggaaactggtcgctttagtattgagttcatgcctccactgacgcttcaggaaaccgactgcgacgatgctcgctcactcaatgaagccattgagtactttgtgacgaaaaacccagagcaatacatgtggaccctgcgtctactgcgtacacaggcggatggcagtaacccatacagtgaaatgcgtgagcatggctttattaaagagaagtga

SEQ ID NO: 3 - DNA, 5395 bp, Artificial Sequence
  Synthetic
  misc_feature: Allelic exchange plasmid to delete lpxL
caaccatcatcgatgaattgcttcgttaatacagatgtaggtgttccacagggtagccagcagcatcctgcgatgcagatccggatgccatttcattacctctttctccgcacccgacatagatccgaagatcagcagttcaacctgttgatagtacgtactaagctctcatgtttcacgtactaagctctcatgtttaacgtactaagctctcatgtttaacgaactaaaccctcatggctaacgtactaagctctcatggctaacgtactaagctctcatgtttcacgtactaagctctcatgtttgaacaataaaattaatataaatcagcaacttaaatagcctctaaggttttaagttttataagaaaaaaaagaatatataaggcttttaaagcttttaaggtttaacggttgtggacaacaagccagggatctgccatttcattacctctttctccgcacccgacatagatccggaacataatggtgcagggcgctgacttccgcgtttccagactttacgaaacacggaaaccgaagaccattcatgttgttgctcaggtcgcagacgttttgcagcagcagtcgcttcacgttcgctcgcgtatcggtgattcattctgctaaccagtaaggcaaccccgccagcctagccgggtcctcaacgacaggagcacgatcatgcgcacccgtggccaggacccaacgctgcccgagatgcgccgcgtgcggctgctggagatggcggacgcgatggatatgttctgccaagggttggtttgcgcattcacaggtcgtggaaacgatagggacggatctgctggcgaaagggggatgtgctgcaaggcgattaagttgggtaacgccagggttttcccagtcacgacgttgtaaaacgacggccagtgaattaattcttgaagacgaaagggcctcgtgatacgcctatttttataggttaatgtcatgataataatggtttcttagagcttacggccagcctcgcagagcaggattcccgttgagcaccgccaggtgcgaataagggacagtgaagaaggaacacccgctcgcgggtgggcctacttcacctatcctgcccggctgacgccgttggatacaccaaggaaagtctacacgaaccctttggcaaaatcctgtatatcgtgcgaaaaaggatggatataccgaaaaaatcgctataatgaccccgaagcagggttatgcagcggaaaagatccgtcgatcgacccaggtggcactttatgacaacttgacggctacatcattcactttttcttcacaaccggcacggaactcgctcgggctggccccggtgcattttttaaatacccgcgagaaatagagttgatcgtcaaaaccaacattgcgaccgacggtggcgataggcatccgggtggtgctcaaaagcagcttcgcctggctgatacgttggtcctcgcgccagcttaagacgctaatccctaactgctggcggaaaagatgtgacagacgcgacggcgacaagcaaacatgctgtgcgacgctggcgatatcaaaattgctgtctgccaggtgatcgctgatgtactgacaagcctcgcgtacccgattatccatcggtggatggagcgactcgttaatcgcttccatgcgccgcagtaacaattgctcaagcagatttatcgccagcagctccgaatagcgcccttccccttgcccggcgttaatgatttgcccaaacaggtcgctgaaatgcggctggtgcgcttcatccgggcgaaagaaccccgtattggcaaatattgacggccagttaagccattcatgccagtaggcgcgcggacgaaagtaaacccactggtgataccattcgcgagcctccggatgacgaccgtagtgatgaatctctcctggcgggaacagcaaaatatcacccggtcggcaaacaaattctcgtccctgatttttcaccaccccctgaccgcgaatggtgagattgagaatataacctttcattcccagcggtcggtcgataaaaaaatcgagataaccgttggcctcaatcggcgttaaacccgccaccagatgggcattaaacgagtatcccggcagcaggggatcattttgcgcttcagccatacttttcatactcccgccattcagagaagaaaccaattgtccatattgcatcagacattgccgtcactgcgtcttttactggctcttctcgctaaccaaaccggtaaccccgcttattaaaagcattctgtaacaaagcgggaccaaagccatgacaaaaacgcgtaacaaaagtgtctataatcacggcagaaaagtccacattgattatttgcacggcgtcacactttgctatgccatagcatttttatccataagattagcggatcctacctgacgctttttatcgcaactctctactgtttctccatacccgtttttttgggaattcgagctctaaggaggttataaaaaatgcagtttaaggtttacacctataaaagagagagccgttatcgtctgtttgtggatgtacagagtgatattattgacacgccggggcgacggatggtgatccccctggccagtgcacgtctgctgtcagataaagtctcccgtgaactttacccggtggtgcatatcggggatgaaagctggcgcatgatgaccaccgatatggccagtgtgccggtctccgttatcggggaagaagtggctgatctcagccaccgcgaaaatgacatcaaaaacgccattaacctgatgttctggggaatataattgatattgccttgctgcaacttggttacgataagcagaaagatatccaccatcaccaatatgcttatggcatgttcagtagtgaatcgagttatcgacagctgggtttaatcgatgagcttggagactacagacactttcagcgtgaggttgggaagatgctactcaatactcccgagcctattgatatgcatatctattttgttatttctcaggagcatcacaaagcggctaatacgctacattaatcctttcactgtgccgcaactgttttcaatagcgtggcacagttttctagcttgtttttccaacacatttttctaacacctttctttatcgtcctttccaaagcgtatgcgctgcattttcgggtaggaaaattctatttattcaaaagttcatgaaagtatgtaggtaatttactctaaccaatgttaacgtgctcaaatcttttgtcgcctttacaatttaattcgaagtcagtttgggttccctgtgtagtgtgtcgaagatccataaaatacccgcgctttaactttttttgaagtgcaaacaatgataaacgtttatgcaattatcattaactttaattacttatagtaccgttcgtatagcatacattatacgaagttattgatgtccggcggtgcttttgccgttacgcaccaccccgtcagtagctgaacaggagggacagctgatagaaacagaagccactggagcacctcaaaaacaccatcatacactaaatcagtaagttggcagcatcacccgacgcactttgcgccgaataaatacctgtgacggaagatcacttcgcagaataaataaatcctggtgtccctgttgataccgggaagccctgggccaacttttggcgaaaatgagacgttgatcggcacgtaagaggttccaactttcaccataatgaaataagatcactaccgggcgtattttttgagttatcgagattttcaggagctaaggaagctaaaatggagaaaaaaatcactggatataccaccgttgatatatcccaatggcatcgtaaagaacattttgaggcatttcagtcagttgctcaatgtacctataaccagaccgttcagctggatattacggcctttttaaagaccgtaaagaaaaataagcacaagttttatccggcctttattcacattcttgcccgcctgatgaatgctcatccggaattccgtatggcaatgaaagacggtgagctggtgatatgggatagtgttcacccttgttacaccgttttccatgagcaaactgaaacgttttcatcgctctggagtgaataccacgacgatttccggcagtttctacacatatattcgcaagatgtggcgtgttacggtgaaaacctggcctatttccctaaagggtttattgagaatatgtttttcgtctcagccaatccctgggtgagtttcaccagttttgatttaaacgtggccaatatggacaacttcttcgcccccgttttcaccatgggcaaatattatacgcaaggcgacaaggtgctgatgccgctggcgattcaggttcatcatgccgtctgtgatggcttccatgtcggcagaatgcttaatgaattacaacagtactgcgatgagtggcagggcggggcgtaatttttttaaggcagttattggtgcccttaaacgcctggtgctacgcctgaataagtgataataagcggatgaatggcagaaattcgaaagcaaattcgacccggtcgtcggttcagggcagggtcgttaaatagccgcttatgtctattgctggtttaccggtttattgactaccggaagcagtgtgaccgtgtgcttctcaaatgcctgaggccagtttgctcaggctctccccgtggaggtaataattgacgatatgatcatttattctgcctcccagagcctgataaaaacggttaataacttcgtatagcatacattatacgaacggtatgaatcgtttttagctgttaatgctaagtagtggtttaacattttgaagcccccaatcgttcacgattattgggggctttttatttggataagtgaaacgatacggggattgagcctcttttctctcgataggctagatcactgaggcctgtcatttctaacctgtttaatctgctattttttttacattcattgggttgtatagtgaatgtactaagcttttctaacaatccgtttttatcaagccaacaccaagaatcgagaactatgccctatgtttgacgagttagcttttgccgggcttctgtttagtccgttggtggtttttatgcctcttgcttttttactgtcatggagtacgcgttttgtgctgcataaatcaggcttatacgcaaaactgtggaaggcaccttggtttgaagtcagcttgtatgtctgttatctcgcgttagtcatttatctatttgggagctaatcatctatgggaaaattcgttcgcatctccctcactcttacgactttggttattgccgttattcttggccattggatttggcaacattatctgtattcgccttggacccgtgatggacgaataag

SEQ ID NO: 4 - DNA, 5395 bp, Artificial Sequence
  Synthetic
  misc_feature: Allelic exchange plasmid to delete lpxM
caaccatcatcgatgaattgcttcgttaatacagatgtaggtgttccacagggtagccagcagcatcctgcgatgcagatccggatgccatttcattacctctttctccgcacccgacatagatccgaagatcagcagttcaacctgttgatagtacgtactaagctctcatgtttcacgtactaagctctcatgtttaacgtactaagctctcatgtttaacgaactaaaccctcatggctaacgtactaagctctcatggctaacgtactaagctctcatgtttcacgtactaagctctcatgtttgaacaataaaattaatataaatcagcaacttaaatagcctctaaggttttaagttttataagaaaaaaaagaatatataaggcttttaaagcttttaaggtttaacggttgtggacaacaagccagggatctgccatttcattacctctttctccgcacccgacatagatccggaacataatggtgcagggcgctgacttccgcgtttccagactttacgaaacacggaaaccgaagaccattcatgttgttgctcaggtcgcagacgttttgcagcagcagtcgcttcacgttcgctcgcgtatcggtgattcattctgctaaccagtaaggcaaccccgccagcctagccgggtcctcaacgacaggagcacgatcatgcgcacccgtggccaggacccaacgctgcccgagatgcgccgcgtgcggctgctggagatggcggacgcgatggatatgttctgccaagggttggtttgcgcattcacaggtcgtggaaacgatagggacggatctgctggcgaaagggggatgtgctgcaaggcgattaagttgggtaacgccagggttttcccagtcacgacgttgtaaaacgacggccagtgaattaattcttgaagacgaaagggcctcgtgatacgcctatttttataggttaatgtcatgataataatggtttcttagagcttacggccagcctcgcagagcaggattcccgttgagcaccgccaggtgcgaataagggacagtgaagaaggaacacccgctcgcgggtgggcctacttcacctatcctgcccggctgacgccgttggatacaccaaggaaagtctacacgaaccctttggcaaaatcctgtatatcgtgcgaaaaaggatggatataccgaaaaaatcgctataatgaccccgaagcagggttatgcagcggaaaagatccgtcgatcgacccaggtggcactttatgacaacttgacggctacatcattcactttttcttcacaaccggcacggaactcgctcgggctggccccggtgcattttttaaatacccgcgagaaatagagttgatcgtcaaaaccaacattgcgaccgacggtggcgataggcatccgggtggtgctcaaaagcagcttcgcctggctgatacgttggtcctcgcgccagcttaagacgctaatccctaactgctggcggaaaagatgtgacagacgcgacggcgacaagcaaacatgctgtgcgacgctggcgatatcaaaattgctgtctgccaggtgatcgctgatgtactgacaagcctcgcgtacccgattatccatcggtggatggagcgactcgttaatcgcttccatgcgccgcagtaacaattgctcaagcagatttatcgccagcagctccgaatagcgcccttccccttgcccggcgttaatgatttgcccaaacaggtcgctgaaatgcggctggtgcgcttcatccgggcgaaagaaccccgtattggcaaatattgacggccagttaagccattcatgccagtaggcgcgcggacgaaagtaaacccactggtgataccattcgcgagcctccggatgacgaccgtagtgatgaatctctcctggcgggaacagcaaaatatcacccggtcggcaaacaaattctcgtccctgatttttcaccaccccctgaccgcgaatggtgagattgagaatataacctttcattcccagcggtcggtcgataaaaaaatcgagataaccgttggcctcaatcggcgttaaacccgccaccagatgggcattaaacgagtatcccggcagcaggggatcattttgcgcttcagccatacttttcatactcccgccattcagagaagaaaccaattgtccatattgcatcagacattgccgtcactgcgtcttttactggctcttctcgctaaccaaaccggtaaccccgcttattaaaagcattctgtaacaaagcgggaccaaagccatgacaaaaacgcgtaacaaaagtgtctataatcacggcagaaaagtccacattgattatttgcacggcgtcacactttgctatgccatagcatttttatccataagattagcggatcctacctgacgctttttatcgcaactctctactgtttctccatacccgtttttttgggaattcgagctctaaggaggttataaaaaatgcagtttaaggtttacacctataaaagagagagccgttatcgtctgtttgtggatgtacagagtgatattattgacacgccggggcgacggatggtgatccccctggccagtgcacgtctgctgtcagataaagtctcccgtgaactttacccggtggtgcatatcggggatgaaagctggcgcatgatgaccaccgatatggccagtgtgccggtctccgttatcggggaagaagtggctgatctcagccaccgcgaaaatgacatcaaaaacgccattaacctgatgttctggggaatataaagcacggtgagaccctatctcaaatcacgggcttccgttacttcaatgtttacggccctcgtgaagaccataaaggaagcatggcatccgttgccttccacctaaataaccagctaaatgcaggtgaaaacccgaaactcttcgcaggtagcgagacctttaaacgtgatttcgtttacgtcggcgatgtatgcaaagtaaatctgtggttcttcgaaaatggcgtatcaggcatttttaactgtggcacaggacgcgcggagtcgtttgaagaggtcgcgaaagcggtgatcactcaccacggaaaaggtgaaatcgaaacgattcctttccctgagcatctaaaaggcgcttaccaagagttcactcaagctgatctgactaagctacgctcagcaggctgcgacgtagaattcaaaacggttgcagaaggtgtctctgaatacctagccatccaaaatcgctaagtatatttgttcgcaataatgaggtggcggtgattatgacctgccacctttactcagcttcaatagcctgtatcatttcctttatctgcatttaaatcactcgtctccatacgcataggtaactagactcccctaccgttcgtatagcatacattatacgaagttattgatgtccggcggtgcttttgccgttacgcaccaccccgtcagtagctgaacaggagggacagctgatagaaacagaagccactggagcacctcaaaaacaccatcatacactaaatcagtaagttggcagcatcacccgacgcactttgcgccgaataaatacctgtgacggaagatcacttcgcagaataaataaatcctggtgtccctgttgataccgggaagccctgggccaacttttggcgaaaatgagacgttgatcggcacgtaagaggttccaactttcaccataatgaaataagatcactaccgggcgtattttttgagttatcgagattttcaggagctaaggaagctaaaatggagaaaaaaatcactggatataccaccgttgatatatcccaatggcatcgtaaagaacattttgaggcatttcagtcagttgctcaatgtacctataaccagaccgttcagctggatattacggcctttttaaagaccgtaaagaaaaataagcacaagttttatccggcctttattcacattcttgcccgcctgatgaatgctcatccggaattccgtatggcaatgaaagacggtgagctggtgatatgggatagtgttcacccttgttacaccgttttccatgagcaaactgaaacgttttcatcgctctggagtgaataccacgacgatttccggcagtttctacacatatattcgcaagatgtggcgtgttacggtgaaaacctggcctatttccctaaagggtttattgagaatatgtttttcgtctcagccaatccctgggtgagtttcaccagttttgatttaaacgtggccaatatggacaacttcttcgcccccgttttcaccatgggcaaatattatacgcaaggcgacaaggtgctgatgccgctggcgattcaggttcatcatgccgtctgtgatggcttccatgtcggcagaatgcttaatgaattacaacagtactgcgatgagtggcagggcggggcgtaatttttttaaggcagttattggtgcccttaaacgcctggtgctacgcctgaataagtgataataagcggatgaatggcagaaattcgaaagcaaattcgacccggtcgtcggttcagggcagggtcgttaaatagccgcttatgtctattgctggtttaccggtttattgactaccggaagcagtgtgaccgtgtgcttctcaaatgcctgaggccagtttgctcaggctctccccgtggaggtaataattgacgatatgatcatttattctgcctcccagagcctgataaaaacggttaataacttcgtatagcatacattatacgaacggtatatcaacatgtcgaaaaacaaaattctaattattggtccttcttgggttggagatatggtgatgtcgcaatccctatacattgttttaaagcaactgaaccctgaaagcgaaattgatgtgattgcacccgggtggtgtaaaccaatcttagagcgtatgcctgaggtgaataaggccattgaaatgccgattgggcatggtgaatttaaccttctggggcggcgtgaaattggtaaaacgctgcgtgagaagaaatacgatcacgcttatatcctgccaaaatcggcgaaatccgctctgataccttggtttgctaacattcctcttcgcaccggctggaaaggcgaaatgcgctatggcttgctgaatgacattcgtcctaacatgaagtcgttccaatacatggtggagcgttatgtggctttggcttatccacaatcggagatggtggactcatcgtcactaggtggattagagacgctgccgcgccctcgcctagctatcaatactgaagagcaacaaaccactatccagaagtttaacctcaataaagaacgctctattattggcttgtgcccaggtgcagaatttggtccggc